European Patent Application EP 4 737 580 A1, published May 6, 2026. Title: MANUFACTURING METHOD OF RESOLVIN D5 FROM DHA-ENHANCED OIL IN A BIOREACTOR BY LIPOXYGENASE. Applicant: KONKUK UNIVERSITY INDUSTRIAL COOPERATION CORP. The sequence listing filed with the application follows.

SEQUENCE LISTING (2 sequences)

SEQ ID NO: 1 - protein, 681 aa, synthetic construct
MRSIPSLPQNDSPAQQELRLATLTQERQVYAYNFDSRLSPLGIAAQVPRQDNFSFVWLDGVATTGLQLLGNVLAIGAKLFDNGEAIQNDAGLSELELRRVEGTYRELTDGFSRLSDRTSRLHQAPRSPAVTLIADVIERPRTLLKAAGQKLEETAGVAIVSELATQAALDAPAIGQDILDLIDTLLKKLLSEAGDLFLKYLGLYGKAASLDNYTAQFSLLQPPSVASNYETDLIFARMRLAGPNPALLQGIAALPEKFPVTDAQYQSVMGSQDTLARAGQEGRLYLLDYAVFQGIPTGQTSGGQKYIEAPLALFAVPAANQADRKLRAVAIQCSQTPGRSNPIFTPADGTSWSLARLHVQVADGNYHELIAHLGLTHLILEEFTLSTHRQLAPQHPLYLLLTPHFQGTLAINNAAETSLIAPGGPVDQLLAGEIKASTQVSIQAVANQSINQSFLPRALAARGVDDASKLPDYPYRDDALLLWNDIRAWVSDYLAIYYNDDAAVRSDYELQAWVTELASPDAGKLKDVTEGGGGIQTFEYLVDLTTYIIFTASVQHAAVNFPQRTVMSYTPALPLAAYAPAPTSVEELPPSTELTHLPPLQMAFLQQAVTFGLGNVYFTRLGGYDTYLREPWFADARVWPALEVFQKRLRATEREIGQRNLSRIPYETLLPTAIPQSINIZ

SEQ ID NO: 2 - DNA, 2043 bp, synthetic construct
  source 1..2043: mol_type = other DNA
atgcgttccattccctccctgccccagaatgactctcccgcccagcaggagctgcgcctcgccacgctcacacaagagcggcaggtctacgcctacaacttcgacagccggctgagtccgctggggatcgcggcccaggtcccccgtcaggacaacttctccttcgtctggttggatggcgtcgccaccaccggcctgcagctgctgggcaacgtgctggccatcggcgcgaagctcttcgacaacggggaggcgatccagaacgacgccggcctgtccgagctggagctccgcagggtcgaggggacctaccgggagctgaccgacggattcagccggctgtcggaccggacctcccggctccaccaggcgccgcgctccccggcggtgacgctcatcgccgatgtcatcgagcgcccccggacgctgctcaaggcggcgggccagaagctggaggagaccgccggtgtcgccatcgtctccgagctcgccacccaggccgcgctggatgcgcccgccatcgggcaggacatcctcgacctcatcgacaccctgttgaagaagctgttgtccgaggccggagatctgttcctgaagtacctggggctgtacggcaaggcggcgtcgctcgacaactacacggcccagttctcgctgctgcagcctccgtcggtcgccagcaattacgagaccgacctcatcttcgcgcgcatgcggctggccgggcccaacccggcgctgctccagggcatcgcggccctccccgagaagttcccggtgacggacgcgcagtaccagtccgtgatgggctcgcaggacaccctggcccgcgcgggccaggaaggtcggctgtacctgctggactacgccgtcttccagggcatccccaccggacagacgtcgggcggacagaagtacatcgaagcgccgctcgccctgttcgccgtgcccgccgcgaaccaggccgaccggaagctgcgcgcggtggccatccagtgctcgcagacgccgggccgctccaaccccatcttcaccccggcggacggcacctcctggagcctggcgcgcctgcacgtgcaggtggcggatggcaactaccacgagctcatcgcgcacctgggcctcacgcacctgattctggaagagttcaccctgtccacgcaccggcagctcgcgccccagcacccgctctacctgctgctgacgccgcacttccagggcaccctggccatcaacaacgccgcggagacgtccctcatcgcgcccggtggcccggtggaccagctgctcgccggtgagatcaaggcctccacccaggtgagcatccaggccgtggccaaccaatccatcaaccagtcgttcctgccccgggcgctggcggcccgcggggtggacgacgcctcgaagctgccggactacccgtaccgcgacgacgcgctgctgctctggaacgacatccgcgcctgggtgagcgactacctggccatctactacaacgatgacgcggcggtgcggagcgactacgagctgcaggcctgggtcacggagctcgccagccccgacgccggcaagctgaaggatgtgacggagggcggagggggcatccagaccttcgagtatctggtggacctgaccacctacatcatcttcacggcgagcgtgcagcacgcggcggtcaacttcccgcagcgcacggtcatgagctacaccccggcgctgccgctggcggcctacgctcccgcgcccacctccgtggaagagctgccgccgagcacggagctgacccacctgccgccgttgcagatggccttcctgcagcaggcggtcaccttcgggctgggcaacgtgtacttcacccggctgggcggctacgacacgtacctgcgcgagccctggttcgcggacgcgcgcgtgtggcccgccctggaggtcttccagaagcgcctgcgcgccacggagcgggagatcggccagcgcaacctgtcgcgcatcccctacgagacgctgctgcccacggcgattccgcagagcatcaacatctaa